European Patent Application EP 4 219 554 A1, published August 2, 2023. Title: CD7-TARGETING HUMANIZED ANTIBODY AND USE THEREOF. Applicant: Bioheng Therapeutics Limited. The sequence listing filed with the application follows.

SEQUENCE LISTING (45 sequences)

SEQ ID NO: 1 - protein, 11 aa, Artificial Sequence
  CDR-L1
RASQSISNNLH

SEQ ID NO: 2 - protein, 7 aa, Artificial Sequence
  CDR-L2
SASQSIS

SEQ ID NO: 3 - protein, 9 aa, Artificial Sequence
  CDR-L3
QQSNSWPYT

SEQ ID NO: 4 - protein, 7 aa, Artificial Sequence
  CDR-H1
GYTFTSY

SEQ ID NO: 5 - protein, 6 aa, Artificial Sequence
  CDR-H2
NPSNGR

SEQ ID NO: 6 - protein, 14 aa, Artificial Sequence
  CDR-H3
GGVYYDLYYYALDY

SEQ ID NO: 7 - protein, 249 aa, Artificial Sequence
  m189
DIELTQSPATLSVTPGDSVSLSCRASQSISNNLHWYQQKSHESPRLLIKSASQSISGIPSRFSGSGSGTDFTLSINSVETEDFGMYFCQQSNSWPYTFGGGTKLEIKRGSTSGSGKPGSGEGSTKGQVQLQESGAELVKPGASVKLSCKASGYTFTSYWMHWVKQRPGQGLEWIGKINPSNGRTNYNEKFKSKATLTVDKSSSTAYMQLSSLTSEDSAVYYCARGGVYYDLYYYALDYWGQGTTVTVSS

SEQ ID NO: 8 - protein, 108 aa, Artificial Sequence
  h189-1 VL
EIVLTQSPATLSLSPGERATLSCRASQSISNNLHWYQQKPGQAPRLLIYSASQSISGIPARFSGSGPGTDFTLTISSLEPEDFAVYYCQQSNSWPYTFGQGTKVEIKR

SEQ ID NO: 9 - protein, 123 aa, Artificial Sequence
  h189-1 VH
QVQLVQSGAEVKKPGASVKVSCKASGYTFTSYYMHWVRQAPGQGLEWMGWINPSNGRTNYAQKFQGRVTMTRDTSISTAYMELSRLRSDDTAVYYCARGGVYYDLYYYALDYWGQGTLVTVSS

SEQ ID NO: 10 - protein, 249 aa, Artificial Sequence
  h189-1 scFv
EIVLTQSPATLSLSPGERATLSCRASQSISNNLHWYQQKPGQAPRLLIYSASQSISGIPARFSGSGPGTDFTLTISSLEPEDFAVYYCQQSNSWPYTFGQGTKVEIKRGSTSGSGKPGSGEGSTKGQVQLVQSGAEVKKPGASVKVSCKASGYTFTSYYMHWVRQAPGQGLEWMGWINPSNGRTNYAQKFQGRVTMTRDTSISTAYMELSRLRSDDTAVYYCARGGVYYDLYYYALDYWGQGTLVTVSS

SEQ ID NO: 11 - protein, 108 aa, Artificial Sequence
  h189-2 VL
DVVMTQSPAFLSVTPGEKVTITCRASQSISNNLHWYQQKPDQAPKLLIKSASQSISGVPSRFSGSGSGTDFTFTISSLEAEDAATYYCQQSNSWPYTFGQGTKVEIKR

SEQ ID NO: 12 - protein, 123 aa, Artificial Sequence; identical to SEQ ID NO: 9
  h189-2 VH

SEQ ID NO: 13 - protein, 249 aa, Artificial Sequence
  h189-2 scFv
DVVMTQSPAFLSVTPGEKVTITCRASQSISNNLHWYQQKPDQAPKLLIKSASQSISGVPSRFSGSGSGTDFTFTISSLEAEDAATYYCQQSNSWPYTFGQGTKVEIKRGSTSGSGKPGSGEGSTKGQVQLVQSGAEVKKPGASVKVSCKASGYTFTSYYMHWVRQAPGQGLEWMGWINPSNGRTNYAQKFQGRVTMTRDTSISTAYMELSRLRSDDTAVYYCARGGVYYDLYYYALDYWGQGTLVTVSS

SEQ ID NO: 14 - protein, 108 aa, Artificial Sequence
  h189-3 VL
DVVMTQSPAFLSVTPGEKVTITCRASQSISNNLHWYQQKPDQAPKLLIKSASQSISGVPSRFSGSGSGTDFTFTISSLEAEDAAMYFCQQSNSWPYTFGQGTKVEIKR

SEQ ID NO: 15 - protein, 123 aa, Artificial Sequence
  h189-3 VH
QVQLVQSGAEVKKPGASVKVSCKASGYTFTSYWMHWVRQAPGQGLEWMGKINPSNGRTNYAQKFQGRVTMTRDTSISTAYMELSRLRSDDTAVYYCARGGVYYDLYYYALDYWGQGTLVTVSS

SEQ ID NO: 16 - protein, 249 aa, Artificial Sequence
  h189-3 scFv
DVVMTQSPAFLSVTPGEKVTITCRASQSISNNLHWYQQKPDQAPKLLIKSASQSISGVPSRFSGSGSGTDFTFTISSLEAEDAAMYFCQQSNSWPYTFGQGTKVEIKRGSTSGSGKPGSGEGSTKGQVQLVQSGAEVKKPGASVKVSCKASGYTFTSYWMHWVRQAPGQGLEWMGKINPSNGRTNYAQKFQGRVTMTRDTSISTAYMELSRLRSDDTAVYYCARGGVYYDLYYYALDYWGQGTLVTVSS

SEQ ID NO: 17 - protein, 108 aa, Artificial Sequence
  h189-4 VL
EIVLTQSPATLSLSPGERATLSCRASQSISNNLHWYQQKPGQAPRLLIKSASQSISGIPARFSGSGPGTDFTLTISSLEPEDFAVYFCQQSNSWPYTFGQGTKVEIKR

SEQ ID NO: 18 - protein, 123 aa, Artificial Sequence; identical to SEQ ID NO: 15
  h189-4 VH

SEQ ID NO: 19 - protein, 249 aa, Artificial Sequence
  h189-4 scFv
EIVLTQSPATLSLSPGERATLSCRASQSISNNLHWYQQKPGQAPRLLIKSASQSISGIPARFSGSGPGTDFTLTISSLEPEDFAVYFCQQSNSWPYTFGQGTKVEIKRGSTSGSGKPGSGEGSTKGQVQLVQSGAEVKKPGASVKVSCKASGYTFTSYWMHWVRQAPGQGLEWMGKINPSNGRTNYAQKFQGRVTMTRDTSISTAYMELSRLRSDDTAVYYCARGGVYYDLYYYALDYWGQGTLVTVSS

SEQ ID NO: 20 - DNA, 747 bp, Artificial Sequence
  h189-1 scFv
gaaattgtgctcactcaaagtcctgcaacccttagcctgtctccaggagagcgagccactctgtcttgcagagccagccaatctatctctaataacctgcactggtatcaacagaagcctggtcaggcacctaggctcctgatatattccgcgtctcagtccatatcaggcatccctgctcgattcagcggctctggtcccggtactgattttacgttgactataagcagtcttgaaccagaggattttgcagtttactattgtcagcagtcaaacagctggccttataccttcggccagggaaccaaggtagaaatcaaacgcggaagtacgtccggctcaggaaagccaggatctggagagggatcaactaagggacaagtgcagctggtgcagtcaggagctgaagttaagaagccaggagcctccgtcaaggtctcctgcaaggccagcgggtatactttcacgtcctattatatgcactgggtgaggcaagctcctggtcagggattggagtggatgggctggatcaacccttcaaacggacgcaccaactacgcacagaaattccaaggtcgggtaaccatgacgagagacacgagtattagcacggcatatatggagttgtctcgactgaggagcgacgacacggccgtgtactattgcgcgcgaggtggggtgtactatgacctgtattattacgcattggactattgggggcagggaacactcgtcactgtttccagc

SEQ ID NO: 21 - DNA, 747 bp, Artificial Sequence
  h189-2 scFv
gatgtcgttatgacgcaaagcccagcctttctctccgtaacgcctggcgaaaaagttacgatcacctgccgggcatctcaaagtatcagtaacaatttgcattggtatcaacagaaacccgaccaagccccaaaactccttatcaagagcgctagtcagagtatctccggcgtcccttctcgattctctggctcaggtagtggaactgatttcaccttcactatatctagtttggaagctgaagacgcggccacttactactgtcagcagtcaaatagttggccctacaccttcggtcaagggacaaaagtcgagatcaaacgaggctcaacctctggtagcgggaagcctggatctggagaaggcagcacaaagggacaggtgcagttggtccaatctggggcggaggttaagaagcctggggcttctgttaaagtgagttgtaaggcatcaggttatactttcacatcctactacatgcactgggttcggcaggctccgggccagggacttgaatggatggggtggattaatccaagcaatggccgcactaactatgctcagaagttccaaggaagggtcacaatgactagagacacttccatatcaaccgcgtatatggaactttcacgacttcgcagcgacgatactgcggtctattattgtgcgcgagggggagtttattatgacctttactactacgcgcttgattattggggacagggtacccttgttaccgtttccagc

SEQ ID NO: 22 - DNA, 747 bp, Artificial Sequence
  h189-3 scFv
gatgtcgttatgacgcaaagcccagcctttctctccgtaacgcctggcgaaaaagttacgatcacctgccgggcatctcaaagtatcagtaacaatttgcattggtatcaacagaaacccgaccaagccccaaaactccttatcaagagcgctagtcagagtatctccggcgtcccttctcgattctctggctcaggtagtggaactgatttcaccttcactatatctagtttggaagctgaagacgcggccatgtacttctgtcagcagtcaaatagttggccctacaccttcggtcaagggacaaaagtcgagatcaaacgaggctcaacctctggtagcgggaagcctggatctggagaaggcagcacaaagggacaggtgcagttggtccaatctggggcggaggttaagaagcctggggcttctgttaaagtgagttgtaaggcatcaggttatactttcacatcctactggatgcactgggttcggcaggctccgggccagggacttgaatggatggggaaaattaatccaagcaatggccgcactaactatgctcagaagttccaaggaagggtcacaatgactagagacacttccatatcaaccgcgtatatggaactttcacgacttcgcagcgacgatactgcggtctattattgtgcgcgagggggagtttattatgacctttactactacgcgcttgattattggggacagggtacccttgttaccgtttccagc

SEQ ID NO: 23 - DNA, 747 bp, Artificial Sequence
  h189-4 scFv
gaaatcgtgttgacacagagccctgcaaccctttcactttccccaggcgaacgcgcgaccctgtcatgccgcgctagtcaaagtatatcaaataacctccactggtatcagcaaaagcctggtcaggccccacgcttgttgatcaaatctgcctctcaaagcatcagtggtattcccgctagattctctggtagcgggcctgggaccgatttcactttgactatctcatctttggaaccggaggatttcgctgtctacttttgccaacagagtaattcatggccttatacgttcggacagggaacgaaggtagagattaaaagaggctctacaagcggttccggtaagccgggctctggggaaggttcaacgaaagggcaagtacagctcgtacagtccggggcagaagttaagaagccgggggcatccgtcaaagtatcatgtaaagcgagtggttatacgttcacaagctactggatgcattgggtacgccaagccccaggccaaggattggaatggatgggtaagattaacccgagcaatggaaggacaaattacgctcaaaagttccagggacgggtcacaatgacgcgcgatacgagcattagcacagcctacatggagctttcccgccttaggtcagatgacactgctgtgtattattgcgccagaggtggagtgtattacgacctctattattacgccctcgactattggggacagggtactcttgttactgtgagtagc

SEQ ID NO: 24 - protein, 25 aa, Artificial Sequence
  CD8alpha transmembrane domain
IYIWAPLAGTCGVLLLSLVITLYCK

SEQ ID NO: 25 - DNA, 75 bp, Artificial Sequence
  CD8alpha transmembrane domain
atctacatctgggcgcccttggccgggacttgtggggtccttctcctgtcactggttatcaccctttactgcaaa

SEQ ID NO: 26 - protein, 27 aa, Artificial Sequence
  CD28 transmembrane domain
FWVLVVVGGVLACYSLLVTVAFIIFWV

SEQ ID NO: 27 - DNA, 81 bp, Artificial Sequence
  CD28 transmembrane domain
ttttgggtcctcgtcgtagttggaggggtacttgcctgttatagcctcctggttaccgtagcatttattatattctgggtg

SEQ ID NO: 28 - protein, 41 aa, Artificial Sequence
  CD28 costimulatory domain
RSKRSRLLHSDYMNMTPRRPGPTRKHYQPYAPPRDFAAYRS

SEQ ID NO: 29 - DNA, 123 bp, Artificial Sequence
  CD28 costimulatory domain
aggagtaagaggagcaggctcctgcacagtgactacatgaacatgactccccgccgccccgggcccacccgcaagcattaccagccctatgccccaccacgcgacttcgcagcctatcgctcc

SEQ ID NO: 30 - protein, 40 aa, Artificial Sequence
  4-1BB costimulatory domain
RGRKKLLYIFKQPFMRPVQTTQEEDGCSCRFPEEEEGGCE

SEQ ID NO: 31 - DNA, 120 bp, Artificial Sequence
  4-1BB costimulatory domain
cggggcagaaagaaactcctgtatatattcaaacaaccatttatgagaccagtacaaactactcaagaggaagatggctgtagctgccgatttccagaagaagaagaaggaggatgtgaa

SEQ ID NO: 32 - protein, 113 aa, Artificial Sequence
  CD3zeta signaling domain
LRVKFSRSADAPAYQQGQNQLYNELNLGRREEYDVLDKRRGRDPEMGGKPRRKNPQEGLYNELQKDKMAEAYSEIGMKGERRRGKGHDGLYQGLSTATKDTYDALHMQALPPR

SEQ ID NO: 33 - DNA, 339 bp, Artificial Sequence
  CD3zeta signaling domain
ctgagagtgaagttcagcaggagcgcagacgcccccgcgtaccagcagggccagaaccagctctataacgagctcaatctaggacgaagagaggagtacgatgttttggacaagagacgtggccgggaccctgagatggggggaaagccgagaaggaagaaccctcaggaaggcctgtacaatgaactgcagaaagataagatggcggaggcctacagtgagattgggatgaaaggcgagcgccggaggggcaaggggcacgatggcctttaccagggtctcagtacagccaccaaggacacctacgacgcccttcacatgcaggccctgccccctcgc

SEQ ID NO: 34 - protein, 114 aa, Artificial Sequence
  CD3zeta signaling domain
LRVKFSRSADAPAYQQGQNQLFNELNLGRREEFDVLDKRRGRDPEMGGKPQRRKNPQEGLYNELQKDKMAEAYSEIGMKGERRRGKGHDGLFQGLSTATKDTFDALHMQALPPR

SEQ ID NO: 35 - DNA, 342 bp, Artificial Sequence
  CD3zeta signaling domain
ctgagagtgaagttcagcaggagcgcagacgcccccgcgtaccagcagggccagaaccagctctttaacgagctcaatctaggacgaagagaggagttcgatgttttggacaagagacgtggccgggaccctgagatggggggaaagccgcagagaaggaagaaccctcaggaaggcctgtacaatgaactgcagaaagataagatggcggaggcctacagtgagattgggatgaaaggcgagcgccggaggggcaaggggcacgatggccttttccagggtctcagtacagccaccaaggacacctttgacgcccttcacatgcaggccctgccccctcgc

SEQ ID NO: 36 - protein, 20 aa, Artificial Sequence
  B2M signal peptide
MSRSVALAVLALLSLSGLEA

SEQ ID NO: 37 - DNA, 60 bp, Artificial Sequence
  B2M signal peptide
atgtcccgctctgttgctttggctgtgctggcccttttgtcccttagcggactggaggcc

SEQ ID NO: 38 - protein, 21 aa, Artificial Sequence
  CD8alpha signal peptide
MALPVTALLLPLALLLHAARP

SEQ ID NO: 39 - DNA, 63 bp, Artificial Sequence
  CD8alpha signal peptide
atggccttaccagtgaccgccttgctcctgccgctggccttgctgctccacgccgccaggccg

SEQ ID NO: 40 - protein, 45 aa, Artificial Sequence
  CD8alpha hinge region
TTTPAPRPPTPAPTIASQPLSLRPEACRPAAGGAVHTRGLDFACD

SEQ ID NO: 41 - DNA, 135 bp, Artificial Sequence
  CD8alpha hinge region
accacgacgccagcgccgcgaccaccaacaccggcgcccaccatcgcgtcgcagcccctgtccctgcgcccagaggcgtgccggccagcggcggggggcgcagtgcacacgagggggctggacttcgcctgtgat

SEQ ID NO: 42 - protein, 39 aa, Artificial Sequence
  CD28 hinge region
IEVMYPPPYLDNEKSNGTIIHVKGKHLCPSPLFPGPSKP

SEQ ID NO: 43 - DNA, 117 bp, Artificial Sequence
  CD28 hinge region
attgaagttatgtatcctcctccttacctagacaatgagaagagcaatggaaccattatccatgtgaaagggaaacacctttgtccaagtcccctatttcccggaccttctaagccc

SEQ ID NO: 44 - protein, 12 aa, Artificial Sequence
  IgG4 hinge region
ESKYGPPCPPCP

SEQ ID NO: 45 - DNA, 36 bp, Artificial Sequence
  IgG4 hinge region
gaaagcaaatacgggccgccgtgtccaccctgtccg